European Patent Application EP 4 748 849 A1, published May 27, 2026. Title: A novel promoter and a method for producing L-arginine using thereof. Applicant: CJ CheilJedang Corporation. Application KR. The sequence listing filed with the application follows.

SEQUENCE LISTING (57 sequences)

SEQ ID NO: 1 - DNA, 40 bp, synthetic construct
  source 1..40: mol_type = other DNA
tgaattcgagctcggtaccccactggtgaactccttgtcc

SEQ ID NO: 2 - DNA, 40 bp, synthetic construct
  source 1..40: mol_type = other DNA
ttgaactaggggcgctttaaaagttttccggtgttgacgg

SEQ ID NO: 3 - DNA, 40 bp, synthetic construct
  source 1..40: mol_type = other DNA
ccgtcaacaccggaaaacttttaaagcgcccctagttcaa

SEQ ID NO: 4 - DNA, 40 bp, synthetic construct
  source 1..40: mol_type = other DNA
gtcgactctagaggatcccccgttgaactgcttgccagcc

SEQ ID NO: 5 - DNA, 40 bp, synthetic construct
  source 1..40: mol_type = other DNA
tgaattcgagctcggtaccctgcggctcgcacggttgctc

SEQ ID NO: 6 - DNA, 40 bp, synthetic construct
  source 1..40: mol_type = other DNA
acggtgcgcaagaagaccacgtcggcagcaaaagcagcct

SEQ ID NO: 7 - DNA, 40 bp, synthetic construct
  source 1..40: mol_type = other DNA
ggctgcttttgctgccgacgtggtcttcttgcgcaccgtg

SEQ ID NO: 8 - DNA, 40 bp, synthetic construct
  source 1..40: mol_type = other DNA
gtcgactctagaggatccccctcttatcaggccaatcggt

SEQ ID NO: 9 - DNA, 42 bp, synthetic construct
  source 1..42: mol_type = other DNA
gtgaattcgagctcggtacccgccccgaaaagccgttaaaag

SEQ ID NO: 10 - DNA, 42 bp, synthetic construct
  source 1..42: mol_type = other DNA
tgccaaaattcacgattattgctcgagtctagagacgggtta

SEQ ID NO: 11 - DNA, 42 bp, synthetic construct
  source 1..42: mol_type = other DNA
ttattggaggagatcaaaacaatgacaatcaaggttgcaatc

SEQ ID NO: 12 - DNA, 42 bp, synthetic construct
  source 1..42: mol_type = other DNA
caggtcggcgtcgcaccttaaggggatcctctagagtcgacc

SEQ ID NO: 13 - DNA, 21 bp, synthetic construct
  source 1..21: mol_type = other DNA
caataatcgtgaattttggca

SEQ ID NO: 14 - DNA, 21 bp, synthetic construct
  source 1..21: mol_type = other DNA
tgttttgatctcctccaataa

SEQ ID NO: 15 - DNA, 150 bp, synthetic construct
  source 1..150: mol_type = other DNA
cctaaatccagcgcgtctgccaattccgccacaagcgcttaatgcgggttttactatacatggtgtagtcccaaattaactaatgcgggtgaccaactgcaccgtaaaaaaaattcgcttatcgtaaatcagcaggtagaataacactct

SEQ ID NO: 16 - DNA, 151 bp, synthetic construct
  source 1..151: mol_type = other DNA
ggcttgttaatcgcttgttaatgcaggcaggtaaggtataacccgagtgttttttcggggaataccaaccctttcaacacaataattttctttaaacatccttgctgtccaccacggctggcaaggaacttaaaatgaaggagcacacctc

SEQ ID NO: 17 - DNA, 151 bp, synthetic construct
  source 1..151: mol_type = other DNA
ctaggtctaaagctaggcgacttgaccaaaattgataggctggggcgggtcttctgaagggcttcggttggggtaagctggcgatctgaaatcgcgctgcattgtggcgtcgaaaagcaaaaaaaatttgtagaagggaagagcgcaccta

SEQ ID NO: 18 - DNA, 320 bp, synthetic construct
  source 1..320: mol_type = other DNA
aagggacggcccgcgcctcgggggggtgtgcgcgggccgtcagtaacccggcaacggggggggggattgtgccggggcaggccacactgtatatcggggccttgcacctgaaattatggcatatcaaacgccacaagacaacatcaaacccgattatttattcgaataacacgaatacttaacagtgtggcaaatgacacttcccgcacgccttctacattcccaatgcgcgaccccagcacgtcacttcaatatcattggtaactttagtttctttctcagtcttggaaagttgccaaaaagcgctaaactatgcggtg

SEQ ID NO: 19 - DNA, 310 bp, synthetic construct
  source 1..310: mol_type = other DNA
aggaggggcctacccgggcagcgccacgccgttcgatccttgactacgcgctacaccctcatctgtgaagagccaccaaacctgggacggttcaagcggcgctaggcgagtctgattgctgcgtcgatctatggggtgagggcagtggccgacatcgcggtccgaactatcgcggtccgaacctaccggagtccgaaagtaccgcggtccgaacctaccggagtccgaaagtaccgcggtccgaacctaccggagtccgaaagtaccgcggtccgaaactatctgatgcgcatcttgtacaatgaggatg

SEQ ID NO: 20 - DNA, 305 bp, synthetic construct
  source 1..305: mol_type = other DNA
cgtctcgaggtgtcttatatatagaggtataggggagaaaaattgagggggagaatccggtcccatcgacttccccatcactgcagtcgccaaaagagtctgtgagtcacatcccaggatgatctcatggcaggaaaagtcggcccgggaaaatacccctgatcttcatcgtgccagagaagggccgcgcatctcgcgagtgcggcagtatccctaaaagttacccccccccgagactataagttcgtgtaactggtgctgttgcaaagttggggcagtaggaagaccggcgtgaaataatcagg

SEQ ID NO: 21 - DNA, 300 bp, synthetic construct
  source 1..300: mol_type = other DNA
tgcggttgtcatggtgacctcttctctgaaacggacggcgggagtaaacgggctgaaaccgattggcccaacctcatggtcagaccacaagaatgtaaggcatgtcacctttgattgtcaatggggtgtagcaaacagggggtggattgtgttgccctcgccttaacgtgtctcctggggtgtggggctgggtgacgtatctgagacgctcggccttgggggggggaaggtacgaatataatttcgaataatgtatgatcaagactcgtctttaaaatggtatttcaaatgtgaggcagt

SEQ ID NO: 22 - DNA, 149 bp, synthetic construct
  source 1..149: mol_type = other DNA
cctaaatccagcgcgtctgccaattccgccacaagcgcttaatgcgggttttactatacatggtgtagtcccaaattaactaatgcgggtgaccaactgcaccgtaaaaaaattcgcttatcgtaaatcagcaggtagaataacactct

SEQ ID NO: 23 - DNA, 151 bp, synthetic construct
  source 1..151: mol_type = other DNA
ggcttgttaatcgcttgttaatgcaggcaggtaaggtataacccgagtgttttttcgaggaataccaaccctttcaacacaataattttctttaaacatccttgctgtccaccacggctggcaaggaacttaaaatgaaggagcacacctc

SEQ ID NO: 24 - DNA, 150 bp, synthetic construct
  source 1..150: mol_type = other DNA
ctaggtctaaagctaggcgacttgaccaaaattgataggctggggcgggtcttctgaagggcttcggttggggtaagctggcgatctgaaatcgcgctgcattgtggcgtcgaaaagcaaaaaaatttgtagaagggaagagcgcaccta

SEQ ID NO: 25 - DNA, 318 bp, synthetic construct
  source 1..318: mol_type = other DNA
aagggacggcccgcgcctcgggggggtgtgcgcgggccgtcagtaacccggcaacggggggggattgtgccggggcaggccacactgtatatcggggccttgcacctgaaattatggcatatcaaacgccacaagacaacatcaaacccgattatttattcgaataacacgaatacttaacagtgtggcaaatgacacttcccgcacgccttctacattcccaatgcgcgaccccagcacgtcacttcaatatcattggtaactttagtttctttctcagtcttggaaagttgccaaaaagcgctaaactatgcggtg

SEQ ID NO: 26 - DNA, 278 bp, synthetic construct
  source 1..278: mol_type = other DNA
aggaggggcctacccgggcagcgccacgccgttcgatccttgactacgcgctacaccctcatctgtgaagagccaccaaacctgggacggttcaagcggcgctaggcgagtctgattgctgcgtcgatctatggggtgagggcagtggccgacatcgcggtccgaactatcgcggtccgaacctaccggagtccgaaagtaccgcggtccgaacctaccggagtccgaaagtaccgcggtccgaaactatctgatgcgcatcttgtacaatgaggatg

SEQ ID NO: 27 - DNA, 306 bp, synthetic construct
  source 1..306: mol_type = other DNA
cgtctcgaggtgtcttatatatagaggtataggggagaaaaattgagggggagaatccggtcccatcgacttccccatcactgcagtcgccaaaagagtctgtgagtcacatcccaggatgatctcatggcaggaaaagtcggcccgggaaaatacccctgatcttcatcgtgccagagaagggccgcgcatctcgcgagtgcggcagtatccctaaaagttaccccccccccgagactataagttcgtgtaactggtgctgttgcaaagttggggcagtaggaagaccggcgtgaaataatcagg

SEQ ID NO: 28 - DNA, 301 bp, synthetic construct
  source 1..301: mol_type = other DNA
tgcggttgtcatggtgacctcttctctgaaacggacggcgggagtaaacgggctgaaaccgattggcccaacctcatggtcagaccacaagaatgtaaggcatgtcacctttgattgtcaatggggtgtagcaaacagggggtggattgtgttgccctcgccttaacgtgtctcctggggtgtggggctgggtgacgtatctgagacgctcggccttggggggggggaaggtacgaatataatttcgaataatgtatgatcaagactcgtctttaaaatggtatttcaaatgtgaggcagt

SEQ ID NO: 29 - DNA, 40 bp, synthetic construct
  source 1..40: mol_type = other DNA
tgaattcgagctcggtacccgtgattcgtattcctcggtg

SEQ ID NO: 30 - DNA, 40 bp, synthetic construct
  source 1..40: mol_type = other DNA
gtcgactctagaggatccccgtcttcttgctctggctgcg

SEQ ID NO: 31 - DNA, 40 bp, synthetic construct
  source 1..40: mol_type = other DNA
tgaattcgagctcggtacccgttgtcatcaccgatacctg

SEQ ID NO: 32 - DNA, 40 bp, synthetic construct
  source 1..40: mol_type = other DNA
gtcgactctagaggatccccgcttcatgtacatgccgttt

SEQ ID NO: 33 - DNA, 40 bp, synthetic construct
  source 1..40: mol_type = other DNA
tgaattcgagctcggtacccagcaccgcttcttcgtgcag

SEQ ID NO: 34 - DNA, 40 bp, synthetic construct
  source 1..40: mol_type = other DNA
gtcgactctagaggatccccagtttcccacctttttgaag

SEQ ID NO: 35 - DNA, 40 bp, synthetic construct
  source 1..40: mol_type = other DNA
tgaattcgagctcggtaccccgatgatggtcttgtccaga

SEQ ID NO: 36 - DNA, 40 bp, synthetic construct
  source 1..40: mol_type = other DNA
gtcgactctagaggatcccctgcctggagatgtccatcaa

SEQ ID NO: 37 - DNA, 40 bp, synthetic construct
  source 1..40: mol_type = other DNA
tgaattcgagctcggtacccccaccagtcaggcccgtgtt

SEQ ID NO: 38 - DNA, 40 bp, synthetic construct
  source 1..40: mol_type = other DNA
gtcgactctagaggatcccctactcagggatatctttcga

SEQ ID NO: 39 - DNA, 40 bp, synthetic construct
  source 1..40: mol_type = other DNA
tgaattcgagctcggtaccctcgccgcgttgtgtaaagaa

SEQ ID NO: 40 - DNA, 40 bp, synthetic construct
  source 1..40: mol_type = other DNA
gtcgactctagaggatccccaggtagcaccacctgccgcc

SEQ ID NO: 41 - DNA, 40 bp, synthetic construct
  source 1..40: mol_type = other DNA
tgaattcgagctcggtacccttctagatctattcgccgat

SEQ ID NO: 42 - DNA, 40 bp, synthetic construct
  source 1..40: mol_type = other DNA
gtcgactctagaggatccccttgaagaccagcgcggcgac

SEQ ID NO: 43 - DNA, 5802 bp, synthetic construct
  source 1..5802: mol_type = other DNA
gttcgcttgctgtccataaaaccgcccagtctagctatcgccatgtaagcccactgcaagctacctgctttctctttgcgcttgcgttttcccttgtccagatagcccagtagctgacattcatccggggtcagcaccgtttctgcggactggctttctacgtgttccgcttcctttagcagcccttgcgccctgagtgcttgcggcagcgtgaagctagcttttatcgccattcgccattcaggctgcgcaactgttgggaagggcgatcggtgcgggcctcttcgctattacgccagctggcgaaagggggatgtgctgcaaggcgattaagttgggtaacgccagggttttcccagtcacgacgttgtaaaacgacggccagtgaattcgagctcggtacccggggatcctctagagtcgacctgcaggcatgcaagcttggcgtaatcatggtcatagctgtttcctgtgtgaaattgttatccgctcacaattccacacaacatacgagccggaagcataaagtgtaaagcctggggtgcctaatgagtgagctaactcacattaattgcgttgcgctcactgcccgctttccagtcgggaaacctgtcgtgccagctgcattaatgaatcggccaacgcgcggggagaggcggtttgcgtattgggcgctcttccgcttcctcgctcactgactcgctgcgctcggtcgttcggctgcggcgagcggtatcagctcactcaaaggcggtaatacggttatccacagaatcaggggataacgcaggaaagaacatgtgagcaaaaggccagcaaaaggccaggaaccgtaaaaaggccgcgttgctggcgtttttccataggctccgcccccctgacgagcatcacaaaaatcgacgctcaagtcagaggtggcgaaacccgacaggactataaagataccaggcgtttccccctggaagctccctcgtgcgctctcctgttccgaccctgccgcttaccggatacctgtccgcctttctcccttcgggaagcgtggcgctttctcaatgctcacgctgtaggtatctcagttcggtgtaggtcgttcgctccaagctgggctgtgtgcacgaaccccccgttcagcccgaccgctgcgccttatccggtaactatcgtcttgagtccaacccggtaagacacgacttatcgccactggcagcagccactggtaacaggattagcagagcgaggtatgtaggcggtgctacagagttcttgaagtggtggcctaactacggctacactagaaggacagtatttggtatctgcgctctgctgaagccagttaccttcggaaaaagagttggtagctcttgatccggcaaacaaaccaccgctggtagcggtggtttttttgtttgcaagcagcagattacgcgcagaaaaaaaggatctcaagaagatcctttgatcttttctacggggtctgacgctcagtggaacgaaaactcacgttaagggattttggtcatgagattatcaaaaaggatcttcacctagatccttttggggtgggcgaagaactccagcatgagatccccgcgctggaggatcatccagccctgatagaaacagaagccactggagcacctcaaaaacaccatcatacactaaatcagtaagttggcagcatcacccgacgcactttgcgccgaataaatacctgtgacggaagatcacttcgcagaataaataaatcctggtgtccctgttgataccgggaagccctgggccaacttttggcgaaaatgagacgttgatcggcacgtaagaggttccaactttcaccataatgaaataagatcactaccgggcgtattttttgagttatcgagattttcaggagctgatagaaacagaagccactggagcacctcaaaaacaccatcatacactaaatcagtaagttggcagcatcacccgacgcactttgcgccgaataaatacctgtgacggaagatcacttcgcagaataaataaatcctggtgtccctgttgataccgggaagccctgggccaacttttggcgaaaatgagacgttgatcggcacgtaagaggttccaactttcaccataatgaaataagatcactaccgggcgtattttttgagttatcgagattttcaggagctctttggcatcgtctctcgcctgtcccctcagttcagtaatttcctgcatttgcctgtttccagtcggtagatattccacaaaacagcagggaagcagcgcttttccgctgcataaccctgcttcggggtcattatagcgattttttcggtatatccatcctttttcgcacgatatacaggattttgccaaagggttcgtgtagactttccttggtgtatccaacggcgtcagccgggcaggataggtgaagtaggcccacccgcgagcgggtgttccttcttcactgtcccttattcgcacctggcggtgctcaacgggaatcctgctctgcgaggctggccggctaccgccggcgtaacagatgagggcaagcggatggctgatgaaaccaagccaaccaggaagggcagcccacctatcaaggtgtactgccttccagacgaacgaagagcgattgaggaaaaggcggcggcggccggcatgagcctgtcggcctacctgctggccgtcggccagggctacaaaatcacgggcgtcgtggactatgagcacgtccgcgagggcgtcccggaaaacgattccgaagcccaacctttcatagaaggcggcggtggaatcgaaatctcgtgatggcaggttgggcgtcgcttggtcggtcatttcgaaaaaggttaggaatacggttagccatttgcctgcttttatatagttcatatgggattcacctttatgttgataagaaataaaagaaaatgccaataggatatcggcattttcttttgcgtttttatttgttaactgttaattgtccttgttcaaggatgctgtctttgacaacagatgttttcttgcctttgatgttcagcaggaagctcggcgcaaacgttgattgtttgtctgcgtagaatcctctgtttgtcatatagcttgtaatcacgacattgtttcctttcgcttgaggtacagcgaagtgtgagtaagtaaaggttacatcgttaggcggatcaagatccatttttaacacaaggccagttttgttcagcggcttgtatgggccagttaaagaattagaaacataaccaagcatgtaaatatcgttagacgtaatgccgtcaatcgtcatttttgatccgcgggagtcagtgaacaggtaccatttgccgttcattttaaagacgttcgcgcgttcaatttcatctgttactgtgttagatgcaatcagcggtttcatcacttttttcagtgtgtaatcatcgtttagctcaatcataccgagagcgccgtttgctaactcagccgtgcgttttttatcgctttgcagaagtttttgactttcttgacggaagaatgatgtgcttttgccatagtatgctttgttaaataaagattcttcgccttggtagccatcttcagttccagtgtttgcttcaaatactaagtatttgtggcctttatcttctacgtagtgaggatctctcagcgtatggttgtcgcctgagctgtagttgccttcatcgatgaactgctgtacattttgatacgtttttccgtcaccgtcaaagattgatttataatcctctacaccgttgatgttcaaagagctgtctgatgctgatacgttaacttgtgcagttgtcagtgtttgtttgccgtaatgtttaccggagaaatcagtgtagaataaacggatttttccgtcagatgtaaatgtggctgaacctgaccattcttgtgtttggtcttttaggatagaatcatttgcatcgaatttgtcgctgtctttaaagacgcggccagcgtttttccagctgtcaatagaagtttcgccgactttttgatagaacatgtaaatcgatgtgtcatccgcatttttaggatctccggctaatgcaaagacgatgtggtagccgtgatagtttgcgacagtgccgtcagcgttttgtaatggccagctgtcccaaacgtccaggccttttgcagaagagatatttttaattgtggacgaatcaaattcagaaacttgatatttttcatttttttgctgttcagggatttgcagcatatcatggcgtgtaatatgggaaatgccgtatgtttccttatatggcttttggttcgtttctttcgcaaacgcttgagttgcgcctcctgccagcagtgcggtagtaaaggttaatactgttgcttgttttgcaaactttttgatgttcatcgttcatgtctccttttttatgtactgtgttagcggtctgcttcttccagccctcctgtttgaagatggcaagttagttacgcacaataaaaaaagacctaaaatatgtaaggggtgacgccaaagtatacactttgccctttacacattttaggtcttgcctgctttatcagtaacaaacccgcgcgatttacttttcgacctcattctattagactctcgtttggattgcaactggtctattttcctcttttgtttgatagaaaatcataaaaggatttgcagactacgggcctaaagaactaaaaaatctatctgtttcttttcattctctgtattttttatagtttctgttgcatgggcataaagttgcctttttaatcacaattcagaaaatatcataatatctcatttcactaaataatagtgaacggcaggtatatgtgatgggttaaaaaggatcaccccagagtcccgctcagaagaactcgtcaagaaggcgatagaaggcgatgcgctgcgaatcgggagcggcgataccgtaaagcacgaggaagcggtcagcccattcgccgccaagctcttcagcaatatcacgggtagccaacgctatgtcctgatagcggtccgccacacccagccggccacagtcgatgaatccagaaaagcggccattttccaccatgatattcggcaagcaggcatcgccatgggtcacgacgagatcctcgccgtcgggcatccgcgccttgagcctggcgaacagttcggctggcgcgagcccctgatgctcttcgtccagatcatcctgatcgacaagaccggcttccatccgagtacgtgctcgctcgatgcgatgtttcgcttggtggtcgaatgggcaggtagccggatcaagcgtatgcagccgccgcattgcatcagccatgatggatactttctcggcaggagcaaggtgagatgacaggagatcctgccccggcacttcgcccaatagcagccagtcccttcccgcttcagtgacaacgtcgagacagctgcgcaaggaacgcccgtcgtggccagccacgatagccgcgctgcctcgtcttggagttcattcagggcaccggacaggtcggtcttgacaaaaagaaccgggcgcccctgcgctgacagccggaacacggcggcatcagagcagccgattgtctgttgtgcccagtcatagccgaatagcctctccacccaagcggccggagaacctgcgtgcaatccatcttgttcaatcatgcgaaacgatcctcatcctgtctcttgatcagatcttgatcccctgcgccatcagatccttggcggcaagaaagccatccagtttactttgcagggcttcccaaccttaccagagggcgccccagctggcaattccg

SEQ ID NO: 44 - DNA, 18 bp, synthetic construct
  source 1..18: mol_type = other DNA
ggtgatcccagcgatact

SEQ ID NO: 45 - DNA, 18 bp, synthetic construct
  source 1..18: mol_type = other DNA
atagggcttcagcaaagc

SEQ ID NO: 46 - DNA, 18 bp, synthetic construct
  source 1..18: mol_type = other DNA
agggtaagaaggctgtgt

SEQ ID NO: 47 - DNA, 18 bp, synthetic construct
  source 1..18: mol_type = other DNA
ggcgatagccttgtcgcg

SEQ ID NO: 48 - DNA, 18 bp, synthetic construct
  source 1..18: mol_type = other DNA
acaggaaggactccagga

SEQ ID NO: 49 - DNA, 18 bp, synthetic construct
  source 1..18: mol_type = other DNA
ctctgtgccttcatccag

SEQ ID NO: 50 - DNA, 18 bp, synthetic construct
  source 1..18: mol_type = other DNA
gggtgttgtccatttgtt

SEQ ID NO: 51 - DNA, 18 bp, synthetic construct
  source 1..18: mol_type = other DNA
ttgctcagcgtggatttt

SEQ ID NO: 52 - DNA, 18 bp, synthetic construct
  source 1..18: mol_type = other DNA
agatgatcacaatggggc

SEQ ID NO: 53 - DNA, 18 bp, synthetic construct
  source 1..18: mol_type = other DNA
ggttgaagatctgtcggg

SEQ ID NO: 54 - DNA, 18 bp, synthetic construct
  source 1..18: mol_type = other DNA
cgtccgctgcaaatatct

SEQ ID NO: 55 - DNA, 18 bp, synthetic construct
  source 1..18: mol_type = other DNA
tataacgttgtccgggct

SEQ ID NO: 56 - DNA, 18 bp, synthetic construct
  source 1..18: mol_type = other DNA
attcttcatcttcgacgg

SEQ ID NO: 57 - DNA, 18 bp, synthetic construct
  source 1..18: mol_type = other DNA
tcaaagtgatgaacaggg